European Patent Specification EP 3 554 639 B1, published August 19, 2026. Title: NOVEL RECOMBINANT PROTEIN UK 114 IN STABLE POLYMER FORM FOR USE IN THE TREATMENT, DIAGNOSIS AND PREVENTION OF MALIGNANT SOLID AND SYSTEMIC TUMOURS. Applicant: Bartorelli Cusani, Alberto. The sequence listing filed with the application follows.

SEQUENCE LISTING (8 sequences)

SEQ ID NO: 1 - protein, 140 aa, Capra hircus
GSHMSSLVRRIISTAKAPAAIGPYSQAVLVDRTIYISGQLGMDPASGQLVPGGVVEEAKQALTNIGEILKAAGCDFTNVVKATVLLADINDFSAVNDVYKQYFQSSFPARAAYQVAALPKGGRVEIEAIAVQGPLTTASL

SEQ ID NO: 2 - DNA, 41 bp, Artificial Sequence
  synthetic primer
agcatattcgactgacatatgtcgtctttggtcagaaggat

SEQ ID NO: 3 - DNA, 41 bp, Artificial Sequence
  Synthetic primer
atcgtcgggctcactcgagctagagtgatgctgtcgtgaga

SEQ ID NO: 4 - DNA, 474 bp, Artificial Sequence
  expression vector
atgggcagcagccatcatcatcatcatcacagcagcggcctggtgccgcgcggcagccatatgtcgtctttggtcagaaggataatcagcacggcgaaagcccccgcggccattggtccctacagtcaggctgtgttagtcgacaggaccatttacatttcaggacagctaggtatggaccctgcaagtggacagcttgtgccaggaggggtggtagaagaggctaaacaggctcttacaaacataggtgaaattctgaaagcagcaggctgtgacttcacgaatgtggtaaaagcaacggttttgctggctgacataaatgacttcagtgctgtcaatgatgtctacaaacaatatttccagagtagttttccggcgagagctgcttaccaggttgctgctttgcccaaaggaggccgtgttgagatcgaagcaatagctgtgcaaggacctctcacgacagcatcactctaa

SEQ ID NO: 5 - protein, 157 aa, Artificial Sequence
  His-tag-fusion protein
MGSSHHHHHHSSGLVPRGSHMSSLVRRIISTAKAPAAIGPYSQAVLVDRTIYISGQLGMDPASGQLVPGGVVEEAKQALTNIGEILKAAGCDFTNVVKATVLLADINDFSAVNDVYKQYFQSSFPARAAYQVAALPKGGRVEIEAIAVQGPLTTASL

SEQ ID NO: 6 - protein, 139 aa, Capra hircus
VPMSSLVRRIISTAKAPAAIGPYSQAVLVDRTIYISGQLGMDPASGQLVPGGVVEEAKQALTNIGEILKAAGCDFTNVVKATVLLADINDFSAVNDVYKQYFQSSFPARAAYQVAALPKGGRVEIEAIAVQGPLTTASL

SEQ ID NO: 7 - protein, 137 aa, Capra hircus
MSSLVRRIISTAKAPAAIGPYSQAVLVDRTIYISGQLGMDPASGQLVPGGVVEEAKQALTNIGEILKAAGCDFTNVVKATVLLADINDFSAVNDVYKQYFQSSFPARAAYQVAALPKGGRVEIEAIAVQGPLTTASL

SEQ ID NO: 8 - protein, 139 aa, Capra hircus
VPMSSLVRRIISTAKAPAAIGPYSQAVLVDRTIYISGQLGMDPASGQLVPGGVVEEAKQALTNIGEILKAAGCDFTNVVKATVLLADINDFSAVNDVYKQYFQSSFPARAAYQVAALPKGGRVEIEAIAVQGPLTTASV